European Patent Specification EP 4 126 945 B1, published April 1, 2026. Title: METHODS AND TREATMENT INVOLVING EXCESS FREE LIGHT. Applicant: AEVI GENOMIC MEDICINE, LLC. The sequence listing filed with the application follows.

SEQUENCE LISTING (83 sequences)

SEQ ID NO: 1 - protein, 300 aa, Homo sapiens
  misc_feature: Human DcR3 amino acid sequence
MRALEGPGLSLLCLVLALPALLPVPAVRGVAETPTYPWRDAETGERLVCAQCPPGTFVQRPCRRDSPTTCGPCPPRHYTQFWNYLERCRYCNVLCGEREEEARACHATHNRACRCRTGFFAHAGFCLEHASCPPGAGVIAPGTPSQNTQCQPCPPGTFSASSSSSEQCQPHRNCTALGLALNVPGSSSHDTLCTSCTGFPLSTRVPGAEECERAVIDFVAFQDISIKRLQRLLQALEAPEGWGPTPRAGRAALQLKLRRRLTELLGAQDGALLVRLLQALRVARMPGLERSVRERFLPVH

SEQ ID NO: 2 - protein, 5 aa, Artificial Sequence
  Synthetic: Heavy Chain (HC) CDR1 antibody F19
GYNWH

SEQ ID NO: 3 - protein, 16 aa, Artificial Sequence
  Synthetic: HC CDR2 antibody F19
EITHSGSTNYNPSLKS

SEQ ID NO: 4 - protein, 14 aa, Artificial Sequence
  Synthetic: HC CDR3 antibody F19
EIAVAGTGYYGMDV

SEQ ID NO: 5 - protein, 11 aa, Artificial Sequence
  Synthetic: LC CDR1 antibody F19
RASQGINSAFA

SEQ ID NO: 6 - protein, 7 aa, Artificial Sequence
  Synthetic: LC CDR2 antibody F19
DASSLES

SEQ ID NO: 7 - protein, 9 aa, Artificial Sequence
  Synthetic: LC CDR3 antibody F19
QQFNSYPLT

SEQ ID NO: 8 - protein, 448 aa, Artificial Sequence
  Synthetic: Heavy chain variable region antibody F19
QVQLQQWGAGLLKPSETLSLTCAVYGGSFSGYNWHWIRQPPGKGLEWIGEITHSGSTNYNPSLKSRVTISVDTSKNQFSLKLSSVTAADTAVYYCVREIAVAGTGYYGMDVWGQGTTVTVSSASTKGPSVFPLAPCSRSTSESTAALGCLVKDYFPEPVTVSWNSGALTSGVHTFPAVLQSSGLYSLSSVVTVPSSSLGTKTYTCNVDHKPSNTKVDKRVESKYGPPCPPCPAPEFEGGPSVFLFPPKPKDTLMISRTPEVTCVVVDVSQEDPEVQFNWYVDGVEVHNAKTKPREEQFNSTYRVVSVLTVLHQDWLNGKEYKCKVSNKGLPSSIEKTISKAKGQPREPQVYTLPPSQEEMTKNQVSLTCLVKGFYPSDIAVEWESNGQPENNYKTTPPVLDSDGSFFLYSRLTVDKSRWQEGNVFSCSVMHEALHNHYTQKSLSLSLG

SEQ ID NO: 9 - protein, 214 aa, Artificial Sequence
  Synthetic: Light chain variable region antibody F19
AIQLTQSPSSLSASVGDRVTITCRASQGINSAFAWYQQKPGKAPKLLIYDASSLESGVPSRFSGSGSGTDFTLTISSLQPEDFATYYCQQFNSYPLTFGGGTKVEIKRTVAAPSVFIFPPSDEQLKSGTASVVCLLNNFYPREAKVQWKVDNALQSGNSQESVTEQDSKDSTYSLSSTLTLSKADYEKHKVYACEVTHQGLSSPVTKSFNRGEC

SEQ ID NO: 10 - protein, 11 aa, Artificial Sequence
  Synthetic: Alternative LC CDR1 antibody F19
RASRGINSAFA

SEQ ID NO: 11 - protein, 7 aa, Artificial Sequence
  Synthetic: Alternative LC CDR2 antibody F19
DASSLES

SEQ ID NO: 12 - protein, 9 aa, Artificial Sequence
  Synthetic: Alternative LC CDR3 antibody F19
QQFNSYPLT

SEQ ID NO: 13 - protein, 11 aa, Artificial Sequence
  Synthetic: Alternative LC CDR1 antibody F19
RVSQGISSYLN

SEQ ID NO: 14 - protein, 7 aa, Artificial Sequence
  Synthetic: Alternative LC CDR2 antibody F19
SASNLQS

SEQ ID NO: 15 - protein, 8 aa, Artificial Sequence
  Synthetic: Alternative LC CDR3 antibody F19
ARTNAPPT

SEQ ID NO: 16 - protein, 11 aa, Artificial Sequence
  Synthetic: Alternative LC CDR1 antibody F19
RMSQGISSYLA

SEQ ID NO: 17 - protein, 7 aa, Artificial Sequence
  Synthetic: Alternative LC CDR2 antibody F19
AASTLQS

SEQ ID NO: 18 - protein, 9 aa, Artificial Sequence
  Synthetic: Alternative LC CDR3 antibody F19
QQYYSFPYT

SEQ ID NO: 19 - protein, 11 aa, Artificial Sequence
  Synthetic: Alternative LC CDR1 antibody F19
RASQGVSSYLA

SEQ ID NO: 20 - protein, 7 aa, Artificial Sequence
  Synthetic: Alternative LC CDR2 antibody F19
DASNRAT

SEQ ID NO: 21 - protein, 8 aa, Artificial Sequence
  Synthetic: Alternative LC CDR3 antibody F19
QQRSNWHP

SEQ ID NO: 22 - protein, 5 aa, Artificial Sequence
  Synthetic: HC CDR1 antibody E1
RFNMN

SEQ ID NO: 23 - protein, 17 aa, Artificial Sequence
  Synthetic: HC CDR2 antibody E1
YISSSSYTIYYADSVKG

SEQ ID NO: 24 - protein, 7 aa, Artificial Sequence
  Synthetic: HC CDR3 antibody E1
SIAAFDY

SEQ ID NO: 25 - protein, 11 aa, Artificial Sequence
  Synthetic: LC CDR1 antibody E1
RASQGISSALA

SEQ ID NO: 26 - protein, 7 aa, Artificial Sequence
  Synthetic: LC CDR2 antibody E1
DASSLES

SEQ ID NO: 27 - protein, 8 aa, Artificial Sequence
  Synthetic: LC CDR3 antibody E1
QQFNSYRT

SEQ ID NO: 28 - protein, 12 aa, Artificial Sequence
  Synthetic: Alternative LC CDR1 antibody E1
RASQSVSSSYLT

SEQ ID NO: 29 - protein, 7 aa, Artificial Sequence
  Synthetic: Alternative LC CDR2 antibody E1
GASSRAT

SEQ ID NO: 30 - protein, 9 aa, Artificial Sequence
  Synthetic: Alternative LC CDR3 antibody E1
QQYGSSMYT

SEQ ID NO: 31 - protein, 12 aa, Artificial Sequence
  Synthetic: Alternative LC CDR1 antibody E1
RASQSVSSSYLA

SEQ ID NO: 32 - protein, 7 aa, Artificial Sequence
  Synthetic: Alternative LC CDR2 antibody E1
GASNRAT

SEQ ID NO: 33 - protein, 9 aa, Artificial Sequence
  Synthetic: Alternative LC CDR3 antibody E1
QQYGSSPWT

SEQ ID NO: 34 - protein, 5 aa, Artificial Sequence
  Synthetic: HC CDR1 antibody E13
NAWMS

SEQ ID NO: 35 - protein, 19 aa, Artificial Sequence
  Synthetic: HC CDR2 antibody E13
RIKSKIDGGTTDYAAPVKG

SEQ ID NO: 36 - protein, 8 aa, Artificial Sequence
  Synthetic: HC CDR3 antibody E13
AMAGAFGF

SEQ ID NO: 37 - protein, 12 aa, Artificial Sequence
  Synthetic: LC CDR1 antibody E13
RASQSVSSSYLA

SEQ ID NO: 38 - protein, 7 aa, Artificial Sequence
  Synthetic: LC CDR2 antibody E13
GASSRAT

SEQ ID NO: 39 - protein, 10 aa, Artificial Sequence
  Synthetic: LC CDR3 antibody E13
QQYGSSPMYT

SEQ ID NO: 40 - protein, 7 aa, Artificial Sequence
  Synthetic: HC CDR1 antibody E63
SGGYYWS

SEQ ID NO: 41 - protein, 16 aa, Artificial Sequence
  Synthetic: HC CDR2 antibody E63
YIYYSGSTNYNPSLKS

SEQ ID NO: 42 - protein, 12 aa, Artificial Sequence
  Synthetic: HC CDR3 antibody E63
WITMFRGVGFDP

SEQ ID NO: 43 - protein, 11 aa, Artificial Sequence
  Synthetic: LC CDR1 antibody E63
RASQSIGSSLH

SEQ ID NO: 44 - protein, 7 aa, Artificial Sequence
  Synthetic: LC CDR2 antibody E63
YASQSFS

SEQ ID NO: 45 - protein, 9 aa, Artificial Sequence
  Synthetic: LC CDR3 antibody E63
RQSSSLPLT

SEQ ID NO: 46 - protein, 5 aa, Artificial Sequence
  Synthetic: HC CDR1 antibody F23
GYYWN

SEQ ID NO: 47 - protein, 11 aa, Artificial Sequence
  Synthetic: HC CDR2 antibody F23
EINQYNPSLKS

SEQ ID NO: 48 - protein, 14 aa, Artificial Sequence
  Synthetic: HC CDR3 antibody F23
EIAIADKGYYGLDV

SEQ ID NO: 49 - protein, 11 aa, Artificial Sequence
  Synthetic: LC CDR1 antibody F23
RASQGISSALA

SEQ ID NO: 50 - protein, 7 aa, Artificial Sequence
  Synthetic: LC CDR2 antibody F23
DASSLES

SEQ ID NO: 51 - protein, 9 aa, Artificial Sequence
  Synthetic: LC CDR3 antibody F23
QQFNSYPLT

SEQ ID NO: 52 - protein, 5 aa, Artificial Sequence
  Synthetic: HC CDR1
SYYIH

SEQ ID NO: 53 - protein, 14 aa, Artificial Sequence
  Synthetic: HC CDR2
PGSDITKYNEKFKG

SEQ ID NO: 54 - protein, 10 aa, Artificial Sequence
  Synthetic: HC CDR3
GISTYSAMDF

SEQ ID NO: 55 - protein, 11 aa, Artificial Sequence
  Synthetic: LC CDR1
KASQDVGTAVA

SEQ ID NO: 56 - protein, 7 aa, Artificial Sequence
  Synthetic: LC CDR2
WASTRHT

SEQ ID NO: 57 - protein, 9 aa, Artificial Sequence
  Synthetic: LC CDR3
QQYSSYPLT

SEQ ID NO: 58 - protein, 122 aa, Artificial Sequence
  Synthetic: HC variable region
QVQLVQSGAEVKKPGASVKVSCKASGYTFTSYYIHWVRQAPGQRLEWMGWIFPGSDITKYNEKFKGRVTITRDTSASTAYMELSSLRSEDTAVYYCAREDYGISTYSAMDFWGQGTLVTVSS

SEQ ID NO: 59 - protein, 108 aa, Artificial Sequence
  Synthetic: LC variable region
DIQLTQSPSFLSASVGDRVTITCKASQDVGTAVAWYQQKPGKAPKLLIYWASTRHTGVPSRFSGSGSGTEFTLTISSLQPEDFATYYCQQYSSYPLTFGQGTKVEIKR

SEQ ID NO: 60 - protein, 5 aa, Artificial Sequence
  Synthetic: HC CDR1 of 18E04
HFDIN

SEQ ID NO: 61 - protein, 17 aa, Artificial Sequence
  Synthetic: HC CDR2 of 18E04
WMNPDSDNTDYAQEFQG

SEQ ID NO: 62 - protein, 7 aa, Artificial Sequence
  Synthetic: HC CDR3 of 18E04
GGTTLDY

SEQ ID NO: 63 - protein, 11 aa, Artificial Sequence
  Synthetic: LC CDR1 of 18E04
SGDALPKKYAY

SEQ ID NO: 64 - protein, 7 aa, Artificial Sequence
  Synthetic: LC CDR2 of 18E04
EDSKRPS

SEQ ID NO: 65 - protein, 11 aa, Artificial Sequence
  Synthetic: LC CDR3 of 18E04
YSTDSSDNHVI

SEQ ID NO: 66 - protein, 5 aa, Artificial Sequence
  Synthetic: HC CDR1 of 98C07
DYYMS

SEQ ID NO: 67 - protein, 16 aa, Artificial Sequence
  Synthetic: HC CDR2 of 98C07
YISRSSFIYYSESVKG

SEQ ID NO: 68 - protein, 8 aa, Artificial Sequence
  Synthetic: HC CDR3 of 98C07
WELSPFDY

SEQ ID NO: 69 - protein, 11 aa, Artificial Sequence
  Synthetic: LC CDR1 of 98C07
RASQGISNYLA

SEQ ID NO: 70 - protein, 7 aa, Artificial Sequence
  Synthetic: LC CDR2 of 98C07
AASSLQS

SEQ ID NO: 71 - protein, 9 aa, Artificial Sequence
  Synthetic: LC CDR3 of 98C07
QQYNTYPFT

SEQ ID NO: 72 - protein, 5 aa, Artificial Sequence
  Synthetic: HC CDR1 of 1C02
YYGIS

SEQ ID NO: 73 - protein, 17 aa, Artificial Sequence
  Synthetic: HC CDR2 of 1C02
WISANSGNTNYAQKFQG

SEQ ID NO: 74 - protein, 8 aa, Artificial Sequence
  Synthetic: HC CDR3 of 1C02
GGVAVLEY

SEQ ID NO: 75 - protein, 11 aa, Artificial Sequence
  Synthetic: LC CDR1 of 1C02
WASQGISSYLA

SEQ ID NO: 76 - protein, 7 aa, Artificial Sequence
  Synthetic: LC CDR2 of 1C02
VASTLQS

SEQ ID NO: 77 - protein, 9 aa, Artificial Sequence
  Synthetic: LC CDR3 of 1C02
QQLKIYPLT

SEQ ID NO: 78 - protein, 5 aa, Artificial Sequence
  Synthetic: HC CDR1 of 1C06
DYYMN

SEQ ID NO: 79 - protein, 17 aa, Artificial Sequence
  Synthetic: HC CDR2 of 1C06
DISSRDNTIYYADSVKG

SEQ ID NO: 80 - protein, 14 aa, Artificial Sequence
  Synthetic: HC CDR3 of 1C06
ARERGFGDYFGMDV

SEQ ID NO: 81 - protein, 11 aa, Artificial Sequence
  Synthetic: LC CDR1 of 1C06
RASQDISSALA

SEQ ID NO: 82 - protein, 7 aa, Artificial Sequence
  Synthetic: LC CDR2 of 1C06
DASSLES

SEQ ID NO: 83 - protein, 9 aa, Artificial Sequence
  Synthetic: LC CDR3 of 1C06
QQFNTYPLT